European Patent Application EP 4 624 571 A1, published October 1, 2025. Title: Antibacterial protein for control of Cutibacterium acnes. Applicant: UAB Nomads. The sequence listing filed with the application follows.

SEQUENCE LISTING (1 sequence)

SEQ ID NO: 1 - protein, 813 aa, Cutibacterium acnes
MADQMVLKTQQWLNSTYGNKTGFGSVQETGNTGWDTINALIRALQIELGITATANNFGSGTQSRFKSRWPNGITQTSGYDNVHGIIQGALWCKGYRAEYGGITLEFTDHVADSIRQMKVDIGLGDTSATVDVELMMALLSMKQFRLLSAYGGKTAIRQAQQAINRGYKNYTGIIPTDGLYGREMNTALIQVLQAIEGYTTAEATGNFGAGTRSKLRTISSGTNQWVWLATVSLVCNGYSILPTSTWNSEISNTLWQFQQAHALPVTGVVDPTTWMSLLTSKGDPNRPCVACDTRFEITDELAGHLKADGYQIVGRYLSEPNQSSKSEADYFKALRTGELERIVGHGLKYFPIFQEYSTELKYFSVENGHRHAKEAQTAAQRLGVPPTVIYFAVDYDATDPQVTSHILPYFKAVTQSLGGGYRVGIYASRNICTRIAQAGYAVASFVSDMSTGFSGNLGFPIPDNWVFDQFHEISGYRGKWDLDRVAYSGRMSADSSVRHAQPVNYDALDFLDLIEALESRFEELRVVYKDYAFGEDPITSGSYVTWVKVPTWRCVLNYLSTVYLKGSAKWSAAAEAYREADAKRLEDDTQASQIISALNKWIRSDRQEWTDPAGGAVDIPHMSVTTLGYINLNPLVPDKWTGWAGDLASALGPIQKVVDLNPGSNIIAIARALVGQGDNYKNHSGLQGLTIPNDLPNNCNYSDLCSDGDAIKLAAMLKGSGADDPNLLSRTLRSYYNNPVSLLQRFKAISESVGASDGGTAKDKFFAEIDGPLDDRYVGLLTDGSNGAYGYSGVEPSEETKRAACQALAEFIY